European Patent Application EP 4 442 698 A1, published October 9, 2024. Title: Modified AAV capsid protein and use thereof. Applicant: CHENGDU ORIGEN BIOTECHNOLOGY CO., LTD. The sequence listing filed with the application follows.

SEQUENCE LISTING (28 sequences)

SEQ ID NO: 1 - protein, 5 aa, synthetic construct
RGNRQ

SEQ ID NO: 2 - protein, 10 aa, synthetic construct
QQNTARGNRQ

SEQ ID NO: 3 - protein, 12 aa, synthetic construct
RGNRQAAQQNTA

SEQ ID NO: 4 - protein, 9 aa, synthetic construct
RGNRQQNTA

SEQ ID NO: 5 - protein, 10 aa, synthetic construct
RGNRQQQNTA

SEQ ID NO: 6 - protein, 5 aa, synthetic construct
SGNTQ

SEQ ID NO: 7 - protein, 10 aa, synthetic construct
RGNQQNTARQ

SEQ ID NO: 8 - protein, 12 aa, synthetic construct
RGNQQPRPTSRQ

SEQ ID NO: 9 - protein, 14 aa, synthetic construct
RGNRQAAQQPTPTS

SEQ ID NO: 10 - protein, 10 aa, synthetic construct
SQSGASNDNH

SEQ ID NO: 11 - protein, 432 aa, synthetic construct
SDTGRPFVEMYSEIPEIIHMTEGRELVIPCRVTSPNITVTLKKFPLDTLIPDGKRIIWDSRKGFIISNATYKEIGLLTCEATVNGHLYKTNYLTHRQTNTIIDVVLSPSHGIELSVGEKLVLNCTARTELNVGIDFNWEYPSSKHQHKKLVNRDLKTQSGSEMKKFLSTLTIDGVTRSDQGLYTCAASSGLMTKKNSTFVRVHEKDKTHTCPPCPAPELLGGPSVFLFPPKPKDTLMISRTPEVTCVVVDVSHEDPEVKFNWYVDGVEVHNAKTKPREEQYNSTYRVVSVLTVLHQDWLNGKEYKCKVSNKALPAPIEKTISKAKGQPREPQVYTLPPSRDELTKNQVSLTCLVKGFYPSDIAVEWESNGQPENNYKTTPPVLDSDGSFFLYSKLTVDKSRWQQGNVFSCSVMHEALHNHYTQKSLSLSPGK

SEQ ID NO: 12 - protein, 526 aa, synthetic construct
GRPFVEMYSEIPEIIHMTEGRELVIPCRVTSPNITVTLKKFPLDTLIPDGKRIIWDSRKGFIISNATYKEIGLLTCEATVNGHLYKTNYLTHRQTNTIIDVVLSPSHGIELSVGEKLVLNCTARTELNVGIDFNWEYPSSKHQHKKLVNRDLKTQSGSEMKKFLSTLTIDGVTRSDQGLYTCAASSGLMTKKNSTFVRVHEKPFVAFGSGMESLVEATVGERVRIPAKYLGYPPPEIKWYKNGIPLESNHTIKAGHVLTIMEVSERDTGNYTVILTNPISKEKQSHVVSLVVYVPPGPGDKTHTCPLCPAPELLGGPSVFLFPPKPKDTLMISRTPEVTCVVVDVSHEDPEVKFNWYVDGVEVHNAKTKPREEQYNSTYRVVSVLTVLHQDWLNGKEYKCKVSNKALPAPIEKTISKAKGQPREPQVYTLPPSRDELTKNQVSLTCLVKGFYPSDIAVEWESNGQPENNYKATPPVLDSDGSFFLYSKLTVDKSRWQQGNVFSCSVMHEALHNHYTQKSLSLSPGK

SEQ ID NO: 13 - protein, 123 aa, synthetic construct [sequence omitted]

SEQ ID NO: 14 - protein, 124 aa, synthetic construct
DIQLTQSPSSLSASVGDRVTITCSASQDISNYLNWYQQKPGKAPKVLIYFTSSLHSGVPSRFSGSGSGTDFTLTISSLQPEDFATYYCQQYSTVPWTFGQGTKVEIKRTVAAPSVFIFPPSDEQ

SEQ ID NO: 15 - protein, 120 aa, synthetic construct
EVQLVESGGGLVQPGGSLRLSCTASGFSLTDYYYMTWVRQAPGKGLEWVGFIDPDDDPYYATWAKGRFTISRDNSKNTLYLQMNSLRAEDTAVYYCAGGDHNSGWGLDIWGQGTLVTVSS

SEQ ID NO: 16 - protein, 112 aa, synthetic construct
MEIVMTQSPSTLSASVGDRVIITCQASEIIHSWLAWYQQKPGKAPKLLIYLASTLASGVPSRFSGSGSGAEFTLTISSLQPDDFATYYCQNVYLASTNGANFGQGTKLTVLG

SEQ ID NO: 17 - protein, 121 aa, synthetic construct [sequence omitted]

SEQ ID NO: 18 - protein, 107 aa, synthetic construct [sequence omitted]

SEQ ID NO: 19 - protein, 12 aa, synthetic construct
RGNRQQQPTPTS

SEQ ID NO: 20 - protein, 9 aa, synthetic construct
RGDLTTPQQ

SEQ ID NO: 21 - protein, 9 aa, synthetic construct
RGDLNTPQQ

SEQ ID NO: 22 - protein, 9 aa, synthetic construct
RGDVSSPQQ

SEQ ID NO: 23 - protein, 1299 aa, synthetic construct
AGCGACACCGGCCGGCCCTTCGTGGAGATGTACAGCGAAATCCCTGAGATCATTCACATGACAGAAGGCCGCGAACTGGTGATTCCCTGCAGGGTTACCAGCCCAAACATCACCGTGACCCTGAAGAAGTTCCCCCTGGACACCCTGATCCCTGACGGCAAACGGATCATCTGGGACTCTAGGAAAGGCTTTATCATCTCCAATGCCACATACAAAGAGATTGGCCTGCTGACCTGCGAGGCTACGGTCAACGGCCACCTGTACAAAACAAATTACCTGACCCACAGACAGACCAACACAATCATCGACGTGGTGCTGAGCCCATCCCATGGCATTGAGCTGTCCGTGGGAGAAAAGCTGGTGCTGAATTGTACGGCTAGAACAGAACTTAACGTGGGCATCGATTTCAACTGGGAGTACCCTAGCTCCAAGCACCAGCATAAAAAGCTGGTGAACCGGGACCTGAAGACCCAGTCCGGCAGTGAGATGAAAAAGTTCTTGAGCACCCTGACCATCGATGGAGTGACCCGAAGCGACCAGGGCCTGTACACCTGTGCCGCCTCCTCTGGGCTGATGACAAAAAAGAACAGCACCTTTGTCAGAGTGCACGAGAAGGATAAAACCCACACCTGCCCTCCTTGTCCCGCTCCTGAGCTGCTGGGGGGACCATCTGTGTTCCTGTTCCCCCCCAAGCCCAAGGATACCCTGATGATCAGCCGAACCCCAGAAGTGACCTGCGTGGTGGTGGACGTGTCCCACGAGGACCCAGAGGTGAAATTCAACTGGTATGTGGACGGCGTGGAGGTGCACAATGCCAAGACCAAACCAAGAGAGGAGCAGTATAACTCCACCTACAGGGTGGTGAGCGTGCTGACTGTGCTGCACCAGGATTGGCTGAACGGCAAGGAGTACAAGTGCAAGGTTAGCAATAAAGCTCTGCCCGCCCCCATCGAAAAGACCATTTCCAAAGCCAAAGGGCAGCCAAGGGAGCCCCAGGTGTACACCCTGCCCCCATCTCGGGACGAGCTGACCAAGAACCAGGTGAGTCTCACATGTCTCGTGAAGGGCTTTTACCCTAGCGACATCGCCGTCGAGTGGGAAAGCAACGGACAGCCTGAGAATAACTATAAGACCACACCCCCCGTGCTGGATTCCGACGGCAGTTTTTTCCTGTACTCTAAGCTGACAGTGGACAAATCCCGCTGGCAGCAGGGCAACGTGTTCAGCTGCTCCGTGATGCACGAGGCCCTGCACAATCACTATACACAGAAGAGCCTGAGCCTGAGCCCCGGGAAGTGA

SEQ ID NO: 24 - protein, 466 aa, synthetic construct
LPAQVAFTPYAPEPGSTCRLREYYDQTAQMCCSKCSPGQHAKVFCTKTSDTVCDSCEDSTYTQLWNWVPECLSCGSRCSSDQVETQACTREQNRICTCRPGWYCALSKQEGCRLCAPLRKCRPGFGVARPGTETSDVVCKPCAPGTFSDTTSSTDICRPHQICNVVAIPGDASMDAVCTSTSPTRSMAPGAVHLPQPVSTRSQHTQPTPEPSTAPSTSFLLPMGPSPPAEGSTGDEPKSCDKTHTCPPCPAPELLGGPSVFLFPPKPKDTLMISRTPEVTCVVVDVSHEDPEVKFNWYVDGVEVHNAKTKPREEQYDSTYRVVSVLTVLHQDWLNGKEYKCKVSNKALPAPIEKTISKAKGQPREPQVYTLPPSREEMTKNQVSLTCLVKGFYPSDIAVEWESNGQPENNYKTTPPVLDSDGSFFLYSKLTVDKSRWQQGNVFSCSVMHEALHNHYTQKSLSLSPG

SEQ ID NO: 25 - DNA, 1401 bp, synthetic construct
  source 1..1401: mol_type = other DNA
ctgcccgcccaagtggccttcaccccctatgcccccgagcccggctccacctgtagactgagagagtactacgatcagaccgctcagatgtgctgcagcaagtgcagccccgggcagcacgccaaggtgttctgcaccaagacaagcgacaccgtgtgcgacagctgcgaggacagcacatacacacaactgtggaactgggtgcccgagtgcctgagctgcggcagcagatgcagcagcgaccaagtggagacccaagcctgcacaagagagcagaacagaatctgcacctgcagacccggctggtactgcgccctgagcaagcaagagggctgcagactgtgcgcccccctgagaaagtgtagacccggctttggcgtggctagacccggcacagaaacaagcgacgtcgtgtgcaaaccttgcgctcccggcaccttcagcgacaccacaagcagcaccgacatctgcagaccccatcagatctgcaacgtggtggccatccccggcgacgctagcatggacgccgtctgcacctccacaagccccacccggagcatggctcctggcgccgtgcatctgcctcagcccgtgagcacccggtcccaacacacacagcctacccccgagcctagcaccgctccctccacatccttcctgctccctatggggcctagcccccctgccgaaggcagcaccggcgacgagcccaagagctgcgataaaacccacacatgccccccctgccccgcccctgaactcctgggcgggcctagcgtgttcctgttcccccccaagcccaaggacaccctgatgatcagcagaacccccgaggtgacctgcgtggtcgtggacgtgagccacgaggaccccgaggtgaagttcaactggtacgtggacggcgtggaggtgcacaacgccaagaccaagcctagagaggagcagtacgacagcacctacagagtcgtgagcgtgctgaccgtgctgcaccaagactggctgaacggcaaggagtacaagtgcaaggtgagcaacaaggccctgcccgctcctatcgagaagaccatcagcaaggccaaggggcagcctagagagccccaagtgtacaccctgccccctagcagagaggagatgaccaagaaccaagtgagcctgacctgcctggtgaagggcttctaccctagcgacatcgccgtggagtgggagagcaacgggcagcccgagaacaactacaagaccaccccccccgtgctggacagcgacggcagcttcttcctgtacagcaagctgaccgtggacaagagcagatggcagcaaggcaacgtgttcagctgcagcgtgatgcacgaggccctgcacaaccactacacacagaagagcctgagcctgagccccggctga

SEQ ID NO: 26 - DNA, 20 bp, synthetic construct
  source 1..20: mol_type = other DNA
cacatgaagcagcacgactt

SEQ ID NO: 27 - DNA, 20 bp, synthetic construct
  source 1..20: mol_type = other DNA
tcgtccttgaagaagatggt

SEQ ID NO: 28 - DNA, 21 bp, synthetic construct
  source 1..21: mol_type = other DNA
agtccgccatgcccgaaggct